European Patent Specification EP 3 693 362 B1, published December 20, 2023. Title: Regulator of parasitic plant germination. Applicant: National University Corporation Nagoya University. The sequence listing filed with the application follows.

SEQUENCE LISTING (11 sequences)

SEQ ID NO: 1 - protein, 272 aa, Striga hermonthica
MGLAQEAHNVRVLGSGPQTVVLAHGFGTDQSVWKYLVPHLVEDYRVVLFDIMGAGTTNPTYFNFERYSSLEGYAGDVIAILEELQISSCVYVGHSVSAMIGVIASVTRPDLFTKLVTVAGSPRYLNDPDYFGGFDLDELHELFEAMKENYKAWCSGFAPLCVGADMESLAVQEFSRTLFNMRPDIALSILQTIFYSDVRPLLPHVTVPCHIIQSVKDLAVPVAVSEYIHQSLGGESILEVMATEGHLPQLSSPDVVVPVLLRHIRYAIARPN

SEQ ID NO: 2 - protein, 285 aa, Striga hermonthica
MEEESESRELKKKSVEAAHNVHILGSGDTTVVLGHGFGTDQSVWKYLVPDLVDDYRVLLYDNMGAGTTNPEYFDFDRYSTLEGHASDLLLILDEFNVRSCIFVGHSLSAMTGALASIFRPDLFQKIIMLSSSPRFLNSADYFGGFEPADIEQLAVAIESNYNSWVSGFAPLVVGGDMDSVAVQEFSRTLFNMRPDIARSVFRMIFSFDIRDYLGRVTVPCHIIQSSKDMAVPVSVSEYIRQRVGGRSVVEVMPTEGHLPQLSAPEVTIPVLLRHIRRDIVAAADK

SEQ ID NO: 3 - protein, 276 aa, Striga hermonthica
MNRVEAAHNVHIVGSGDTTVVLGHGFGTDQSVWKHLVPYLVDSYRVLLYDNMGAGTTNPEYFHFERYSTLQGYAHDLLVILHEFNIRSCIFVGHSLSAMTGAIASIIRPDLFQKIVMLSASPRFLNTADYLGGFEPADVEQLAGAIEANYKSWVSGFAPMVVGGDMDSVAVQEFSRTLFNMRPDIARSVFRTIFTSDLRDYLGRVTVPCHIIQSSRDMAVPVSVAEYIHNRVGGRSVVEVMNTEGHLPQLSAPEVAIPVLLRHIKNDIDCLGGRRF

SEQ ID NO: 4 - protein, 271 aa, Striga hermonthica
MSTVGSAHNVRVLGSGETTVVLGHGFGTDQSVWKQLVPYLTDEYRVLLYDNMGAGTTNPDCYDFERYSSLEGHSNDLIAILDDFHVTKCIYVGHSLSSMAAAVSSIFRPDLFRKVVMISATPRITNTEDYYGGFEQEEINQMNTAMEENFKTMMMGFAPIVVGGDLESDAIQEFSRTLFNMRPDIALSICRMISGLDLRPYLGLIVVPCHIIQSSKDMLVPVAVAEYLHKNLGGKSVVELIPTEGHLPHLSAPELTIPVLVRHIKHDIADD

SEQ ID NO: 5 - protein, 271 aa, Striga hermonthica
MSTVGSAHNVTVLGSGETTVVLGHGFGTDQSVWKYLVPHLTDDYRVLLYDNMGAGTTDPNLYDFERYSSLEGHSQDLIAILEEFHVTKCIFVGHSLSSMVGAVSSIFRPDLFRKIVMISACPRVANADDYYGGFEEEDVNQLYGAMEENFQTMMTGYAPIVVGGDLESEAMQEFSRTLFNMRPDIALSICRMISGYDLRPYLGLVVIPCHIIQSSKDKLVPVAVAEYLHRNFGGKSVVELIPTEGHLPHLSAPDITIPVLIRHINQDIADD

SEQ ID NO: 6 - protein, 271 aa, Striga hermonthica
MGTVGAAHNVNVLGSGGTTVVLGHGFGTDQSVWKHLVPHLVDEYRVLLYDNMGAGTTNPDYFDFERYSTLEGYAYDLIAILEEFQVDKCIYVGHSLSSMVAAIASIFRPDLFHKLIMISATPRMMNTDNYFGGFEQEELNQLQAAMEENYASLVSGFAPLMLGCDLDSPVMQEFSRTLFSIRPDIAVNVVRTIHNLDLRPYLGHVTVPCHIIQSSKDIAVPVVVAEYLHRNLGGKSVVELMPTEGHIPHLSSPEVTIPVILRHIKYDIVDN

SEQ ID NO: 7 - protein, 271 aa, Striga hermonthica
MSSIGLAHNVTILGSGETTVVLGHGYGTDQSVWKLLVPYLVDDYKVLLYDHMGAGTTNPDYFDFDRYSSLEGYSYDLIAILEEFQVSKCIYVGHSMSSMAAAVASIFRPDLFHKLVMISPTPRLINTEEYYGGFEQKVMDETLRSLDENFKSLSLGTAPLLLACDLESAAMQEYCRTLFNMRPDIACCITRMICGLDLRPYLGHVTVPCHIIQSSNDIMVPVAVGEYLRKNLGGPSVVEVMPTEGHLPHLSMPEVTIPVVLRHIRQDITDH

SEQ ID NO: 8 - protein, 272 aa, Striga hermonthica
MNNSVGSTHNVTILGSGETTVVLSHGYGTDQSVWKLFVPHLVDDYRVLLYDNMGAGTTNPDYFDFERYSSLEGYSYDLIAILDEFHVSKCIFVGHSMSAMAAAVASIFRPDLFHKLIMISPSPRLANAEDYYGGLEQKEIDEVVGSMEENYRSMALGSAPLLLACDLESAAVQEYCRTLFNMRPDISCCMARMIFGLDLRPYLCHVTVPCHILQSSNDVMVPVAVVEYLSKNLGGPSVVEVMPTEGHLPHLSAPEVTIPVVLRHIRHDIADQ

SEQ ID NO: 9 - protein, 271 aa, Striga hermonthica
MSTVGAAHNVTVLGSGETTVVLGHGFGTDQSVWRHLVPYLVDEYKVLLYDNMGAGTTNPDYFDFERYATLEGYTYDLIAILDEFQVSSCIYVGHSMSAMAAVVASIFRPDLFRKIVMISSTPRLSNTKDYYGGFEQHELDELSAAVEHNYKAMASGYAPLIVGGDLESSAIQEFSRTLFNVRPDIGLSVCRMVNSFDLRPYLSQVTVPCHIIQSSKDTMVPVVMGEYLRRRLGGKTVVEVLPTEGHLPHLSAPEITVPALVRHIRQDIADE

SEQ ID NO: 10 - protein, 268 aa, Striga hermonthica
MNKVGSAHNVTVLGSGETTVVLGHGVCSDQSVWKHLVPHLVDDYTVILYDNIGAGTTDPNLYDFKRYSSIDGYVDDLIAILDELKVEECIFVGHSLSPIVAAIASISRPKLFRKVIMISATPRMANSEGYYGGIDQETIDHIMATFEKNPTSFYTGLAELMVGGSPDSVAVKEFKRTMVMERLDIALHRAGWIYSYDLRPYLSQITVPCHIIHSSKDASVPVEVAEYIHRSLGGRSVLELIPTEGHLPHLSSPELTNPVLLRHIRQDI

SEQ ID NO: 11 - protein, 268 aa, Striga hermonthica
MNKIVSAHNVTVLGSGMTTVVLGHGAGCDQSVWKHLVPHLVDDYTVILYDDIGAGTTDPNLYDFKRYSSIDGYVEDLIAILDELKVEGCIFVGHSLSPLVAAIASISTPKLFRKVIMIATTPRMGNSEDYYGGTDQETMDHMLAALEKNPTSFYADTAKLMVGGSPDSVAVEEFKRTMTMERPDIVLNRGRLIFSYDLRPYLSQITVPCHIIQSSKDPVLPVEVAEYIHRSLGGRSVMELIPTEGHLPHLSSPELTNPVLLRHIRQDI